European Patent Specification EP 4 308 135 B1, published December 3, 2025. Title: THERAPEUTIC USE OF ENGINEERED POSTBIOTICS COMPRISING BACTERIOCINS AND/OR ENDOLYSINS. Applicant: ELIGO BIOSCIENCE. The sequence listing filed with the application follows.

SEQUENCE LISTING (1 sequence)

SEQ ID NO: 1 - protein, 247 aa, Staphylococcus simulans
MAATHEHSAQWLNNYKKGYGYGPYPLGINGGMHYGVDFFMNIGTPVKAISSGKIVEAGWSNYGGGNQIGLIENDGVHRQWYMHLSKYNVKVGDYVKAGQIIGWSGSTGYSTAPHLHFQRMVNSFSNSTAQDPMPFLKSAGYGKAGGTVTPTPNTGWKTNKYGTLYKSESASFTPNTDIITRTTGPFRSMPQSGVLKAGQTIHYDEVMKQDGHVWVGYTGNSGQRIYLPVRTWNKSTNTLGVLWGTIK